European Patent Application EP 4 245 849 A1, published September 20, 2023. Title: NOVEL BRANCHED-CHAIN AMINO ACID AMINOTRANSFERASE VARIANT AND METHOD FOR PRODUCING ISOLEUCINE USING THE SAME. Applicant: CJ CheilJedang Corporation. The sequence listing filed with the application follows.

SEQUENCE LISTING (37 sequences)

SEQ ID NO: 1 - protein, 309 aa, Unknown
  ilvE
MTTKKADYIWFNGEMVRWEDAKVHVMSHALHYGTSVFEGIRCYDSHKGPVVFRHREHMQRLHDSAKIYRFPVSQSIDELMEACRDVIRKNNLTSAYIRPLIFVGDVGMGVNPPAGYSTDVIIAAFPWGAYLGAEALEQGIDAMVSSWNRAAPNTIPTAAKAGGNYLSSLLVGSEARRHGYQEGIALDVNGYISEGAGENLFEVKDGVLFTPPFTSSALPGITRDAIIKLAKELGIEVREQVLSRESLYLADEVFMSGTAAEITPVRSVDGIQVGEGRCGPVTKRIQQAFFGLFTGETEDKWGWLDQVNQ

SEQ ID NO: 2 - protein, 309 aa, Unknown
  ilvE
MTTKKADYIWFNGEMVRWEDAKVHVMSHALLYGTSVFEGIRCYDSHKGPVVFRHREHMQRLHDSAKIYRFPVSQSIDELMEACRDVIRKNNLTSAYIRPLIFVGDVGMGVNPPAGYSTDVIIAAFPWGAYLGAEALEQGIDAMVSSWNRAAPNTIPTAAKAGGNYLSSLLVGSEARRHGYQEGIALDVNGYISEGAGENLFEVKDGVLFTPPFTSSALPGITRDAIIKLAKELGIEVREQVLSRESLYLADEVFMSGTAAEITPVRSVDGIQVGEGRCGPVTKRIQQAFFGLFTGETEDKWGWLDQVNQ

SEQ ID NO: 3 - protein, 309 aa, Unknown
  ilvE
MTTKKADYIWFNGEMVRWEDAKVHVMSHALHYGTSVFEGIRCYDSHKGPVVFRHREHMQRLHDSAKIYRFPVSQSIDELMEACRDVIRKNNLTSAYIIPLIFVGDVGMGVNPPAGYSTDVIIAAFPWGAYLGAEALEQGIDAMVSSWNRAAPNTIPTAAKAGGNYLSSLLVGSEARRHGYQEGIALDVNGYISEGAGENLFEVKDGVLFTPPFTSSALPGITRDAIIKLAKELGIEVREQVLSRESLYLADEVFMSGTAAEITPVRSVDGIQVGEGRCGPVTKRIQQAFFGLFTGETEDKWGWLDQVNQ

SEQ ID NO: 4 - protein, 309 aa, Unknown
  ilvE
MTTKKADYIWFNGEMVRWEDAKVHVMSHALHYGTSVFEGIRCYDSHKGPVVFRHREHMQRLHDSAKIYRFPVSQSIDELMEACRDVIRKNNLTSAYIRPLIFVGDVGMGVNPPAGYSTDVIIAAFPWGAYLGAEALEQGIDAMVSSWNRAAPNTIPTAAKAGGNYLSSLLVGSEARRHGYQEGIALDVNGYISEGAGENLFEVKDGVLFTPPFTSSALPGITRDAIIKLAKELGIEVREQVLSRESLYLADEVFMVGTAAEITPVRSVDGIQVGEGRCGPVTKRIQQAFFGLFTGETEDKWGWLDQVNQ

SEQ ID NO: 5 - protein, 309 aa, Unknown
  ilvE
MTTKKADYIWFNGEMVRWEDAKVHVMSHALLYGTSVFEGIRCYDSHKGPVVFRHREHMQRLHDSAKIYRFPVSQSIDELMEACRDVIRKNNLTSAYIIPLIFVGDVGMGVNPPAGYSTDVIIAAFPWGAYLGAEALEQGIDAMVSSWNRAAPNTIPTAAKAGGNYLSSLLVGSEARRHGYQEGIALDVNGYISEGAGENLFEVKDGVLFTPPFTSSALPGITRDAIIKLAKELGIEVREQVLSRESLYLADEVFMSGTAAEITPVRSVDGIQVGEGRCGPVTKRIQQAFFGLFTGETEDKWGWLDQVNQ

SEQ ID NO: 6 - protein, 309 aa, Unknown
  ilvE
MTTKKADYIWFNGEMVRWEDAKVHVMSHALLYGTSVFEGIRCYDSHKGPVVFRHREHMQRLHDSAKIYRFPVSQSIDELMEACRDVIRKNNLTSAYIRPLIFVGDVGMGVNPPAGYSTDVIIAAFPWGAYLGAEALEQGIDAMVSSWNRAAPNTIPTAAKAGGNYLSSLLVGSEARRHGYQEGIALDVNGYISEGAGENLFEVKDGVLFTPPFTSSALPGITRDAIIKLAKELGIEVREQVLSRESLYLADEVFMVGTAAEITPVRSVDGIQVGEGRCGPVTKRIQQAFFGLFTGETEDKWGWLDQVNQ

SEQ ID NO: 7 - protein, 309 aa, Unknown
  ilvE
MTTKKADYIWFNGEMVRWEDAKVHVMSHALHYGTSVFEGIRCYDSHKGPVVFRHREHMQRLHDSAKIYRFPVSQSIDELMEACRDVIRKNNLTSAYIIPLIFVGDVGMGVNPPAGYSTDVIIAAFPWGAYLGAEALEQGIDAMVSSWNRAAPNTIPTAAKAGGNYLSSLLVGSEARRHGYQEGIALDVNGYISEGAGENLFEVKDGVLFTPPFTSSALPGITRDAIIKLAKELGIEVREQVLSRESLYLADEVFMVGTAAEITPVRSVDGIQVGEGRCGPVTKRIQQAFFGLFTGETEDKWGWLDQVNQ

SEQ ID NO: 8 - DNA, 41 bp, Artificial Sequence
  primer
gaattcgagctcggtacccagacatccttgtcgtccttgcc

SEQ ID NO: 9 - DNA, 40 bp, Artificial Sequence
  primer
ccctcaaatggaattggttagtcagccccattttatggga

SEQ ID NO: 10 - DNA, 24 bp, Artificial Sequence
  primer
accaattccatttgagggcgctca

SEQ ID NO: 11 - DNA, 40 bp, Artificial Sequence
  primer
cagctttcttcgtggtcatgatttcctcgttcccatctcg

SEQ ID NO: 12 - DNA, 44 bp, Artificial Sequence
  primer
gttagatcaagttaatcaataaatcaaccggttttaagaccccg

SEQ ID NO: 13 - DNA, 40 bp, Artificial Sequence
  primer
gtcgactctagaggatcccccctggatcgatctcagatac

SEQ ID NO: 14 - DNA, 25 bp, Artificial Sequence
  primer
atgaccacgaagaaagctgattaca

SEQ ID NO: 15 - DNA, 26 bp, Artificial Sequence
  primer
ttattgattaacttgatctaaccagc

SEQ ID NO: 16 - DNA, 1338 bp, Unknown
  hom
atgacctcagcatctgccccaagctttaaccccggcaagggtcccggctcagcagtcggaattgcccttttaggattcggaacagtcggcactgaggtgatgcgtctgatgaccgagtacggtgatgaacttgcgcaccgcattggtggcccactggaggttcgtggcattgctgtttctgatatctcaaagccacgtgaaggcgttgcacctgagctgctcactgaggacgcttttgcactcatcgagcgcgaggatgttgacatcgtcgttgaggttatcggcggcattgagtacccacgtgaggtagttctcgcagctctgaaggccggcaagtctgttgttaccgccaataaggctcttgttgcagctcactctgctgagcttgctgatgcagcggaagccgcaaacgttgacctgtacttcgaggctgctgttgcaggcgcaattccagtggttggcccactgcgtcgctccctggctggcgatcagatccagtctgtgatgggcatcgttaacggcaccaccaacttcatcttggacgccatggattccaccggcgctgactatgcagattctttggctgaggcaactcgtttgggttacgccgaagctgatccaactgcagacgtcgaaggccatgacgccgcatccaaggctgcaattttggcatccatcgctttccacacccgtgttaccgcggatgatgtgtactgcgaaggtatcagcaacatcagcgctgccgacattgaggcagcacagcaggcaggccacaccatcaagttgttggccatctgtgagaagttcaccaacaaggaaggaaagtcggctatttctgctcgcgtgcacccgactctattacctgtgtcccacccactggcgtcggtaaacaagtcctttaatgcaatctttgttgaagcagaagcagctggtcgcctgatgttctacggaaacggtgcaggtggcgcgccaaccgcgtctgctgtgcttggcgacgtcgttggtgccgcacgaaacaaggtgcacggtggccgtgctccaggtgagtccacctacgctaacctgccgatcgctgatttcggtgagaccaccactcgttaccacctcgacatggatgtggaagatcgcgtgggggttttggctgaattggctagcctgttctctgagcaaggaatctccctgcgtacaatccgacaggaagagcgcgatgatgatgcacatctgatcgtggtcacccactctgcgctggaatctgatctttcccgcaccgttgaactgctgaaggctaagcctgttgttaaggcaatcaacagtgtgatccgcctcgaaagggactaa

SEQ ID NO: 17 - DNA, 35 bp, Artificial Sequence
  primer
tcgagctcggtaccccgcttttgcactcatcgagc

SEQ ID NO: 18 - DNA, 23 bp, Artificial Sequence
  primer
cacgatcagatgtgcatcatcat

SEQ ID NO: 19 - DNA, 23 bp, Artificial Sequence
  primer
atgatgatgcacatctgatcgtg

SEQ ID NO: 20 - DNA, 35 bp, Artificial Sequence
  primer
ctctagaggatccccgagcatcttccaaaaccttg

SEQ ID NO: 21 - DNA, 1311 bp, Artificial Sequence
  ilvA
atgagtgaaacatacgtgtctgagaaaagtccaggagtgatggctagcggagcggagctgattcgtgccgccgacattcaaacggcgcaggcacgaatttcctccgtcattgcaccaactccattgcagtattgccctcgtctttctgaggaaaccggagcggaaatctaccttaagcgtgaggatctgcaggatgttcgttcctacaagatccgcggtgcgctgaactctggagcgcagctcactcaggagcagcgcgatgcaggtatcgttgccgcatctgcaggtaaccatgcccagggcgtggcctatgtgtgcaagtccttgggcgttcagggacgcatctatgttcctgtgcagactccaaagcaaaagcgtgaccgcatcatggttcacggcggagagtttgtctccttggtggtcactggcaataacttcgacgaagcatcggctgcagcgcatgaagatgcagagcgcaccggcgcaacgctgatcgagcctttcgatgctcgcaacaccgtcatcggtcagggtacagtggctgctgagatcttgtcgcagctgacttccatgggcaagagtgcagatcacgtgatggttccagtcggcggtggcggacttcttgcaggtgtggtcagctacatggctgatatggcacctcgcactgcgatcgttggtatcgaaccagcgggagcagcatccatgcaggctgcattgcacaatggtggaccaatcactttggagactgttgatccctttgtggacggcgcagcagtcaaacgtgtcggagatctcaactacaccatcgtggagaagaaccagggtcgcgtgcacatgatgagcgcgaccgagggcgctgtgtgtactgagatgctcgatctttaccaaaacgaaggcatcatcgcggagcctgctggcgcgctgtctatcgctgggttgaaggaaatgtcctttgcacctggttctgtcgtggtgtgcatcatctctggtggcaacaacgatgtgctgcgttatgcggaaatcgctgagcgctccttggtgcaccgcggtttgaagcactacttcttggtgaacttcccgcaaaagcctggtcagttgcgtcacttcctggaagatatcctgggaccggatgatgacatcgcgctggcagagtacctcaagcgcaacaaccgtgagaccggtactgcgttggtgggtattcacttgagtgaagcatcaggattggattctttgctggaacgtatggaggaatcggcaattgattcccgtcgcctcgagccgggcacccctgagtacgaatacttgacctaa

SEQ ID NO: 22 - DNA, 35 bp, Artificial Sequence
  primer
tcgagctcggtacccatgagtgaaacatacgtgtc

SEQ ID NO: 23 - DNA, 39 bp, Artificial Sequence
  primer
gcgcttgaggtactctgccagcgcgatgtcatcatccgg

SEQ ID NO: 24 - DNA, 39 bp, Artificial Sequence
  primer
ccggatgatgacatcgcgctggcagagtacctcaagcgc

SEQ ID NO: 25 - DNA, 34 bp, Artificial Sequence
  primer
ctctagaggatcccccgtcaccgacacctccaca

SEQ ID NO: 26 - DNA, 23 bp, Artificial Sequence
  primer
gagtcgtagcaacggatgccttc

SEQ ID NO: 27 - DNA, 22 bp, Artificial Sequence
  primer
ggcatccgttgctacgactcgc

SEQ ID NO: 28 - DNA, 23 bp, Artificial Sequence
  primer
tgggagtaaacccgccagcggga

SEQ ID NO: 29 - DNA, 23 bp, Artificial Sequence
  primer
tcccgctggcgggtttactccca

SEQ ID NO: 30 - DNA, 930 bp, Unknown
  ilvE
atgaccacgaagaaagctgattacatttggttcaatggggagatggttcgctgggaagacgcgaaggtgcatgtgatgtcgcacgcgctgcactatggcacttcggtttttgaaggcatccgttgctacgactcgcacaaaggaccggttgtattccgccatcgtgagcatatgcagcgtctgcatgactccgccaaaatctatcgcttcccggtttcgcagagcattgatgagctgatggaagcttgtcgtgacgtgatccgcaaaaacaatctcaccagcgcctatatccgtccgctgatcttcgtcggtgatgttggcatgggagtaaacccgccagcgggatactcaaccgacgtgattatcgctgctttcccgtggggagcgtatctgggcgcagaagcgctggagcaggggatcgatgcgatggtttcctcctggaaccgcgcagcaccaaacaccatcccgacggcggcaaaagccggtggtaactacctctcttccctgctggtgggtagcgaagcgcgccgccacggttatcaggaaggtatcgcgctggatgtgaacggttatatctctgaaggcgcaggcgaaaacctgtttgaagtgaaagatggtgtgctgttcaccccaccgttcacctcctccgcgctgccgggtattacccgtgatgccatcatcaaactggcgaaagagctgggaattgaagtacgtgagcaggtgctgtcgcgcgaatccctgtacctggcggatgaagtgtttatgtccggtacggcggcagaaatcacgccagtgcgcagcgtagacggtattcaggttggcgaaggccgttgtggcccggttaccaaacgcattcagcaagccttcttcggcctcttcactggcgaaaccgaagataaatggggctggttagatcaagttaatcaataa

SEQ ID NO: 31 - DNA, 930 bp, Unknown
  ilvE
atgaccacgaagaaagctgattacatttggttcaatggggagatggttcgctgggaagacgcgaaggtgcatgtgatgtcgcacgcgctgctgtatggcacttcggtttttgaaggcatccgttgctacgactcgcacaaaggaccggttgtattccgccatcgtgagcatatgcagcgtctgcatgactccgccaaaatctatcgcttcccggtttcgcagagcattgatgagctgatggaagcttgtcgtgacgtgatccgcaaaaacaatctcaccagcgcctatatccgtccgctgatcttcgtcggtgatgttggcatgggagtaaacccgccagcgggatactcaaccgacgtgattatcgctgctttcccgtggggagcgtatctgggcgcagaagcgctggagcaggggatcgatgcgatggtttcctcctggaaccgcgcagcaccaaacaccatcccgacggcggcaaaagccggtggtaactacctctcttccctgctggtgggtagcgaagcgcgccgccacggttatcaggaaggtatcgcgctggatgtgaacggttatatctctgaaggcgcaggcgaaaacctgtttgaagtgaaagatggtgtgctgttcaccccaccgttcacctcctccgcgctgccgggtattacccgtgatgccatcatcaaactggcgaaagagctgggaattgaagtacgtgagcaggtgctgtcgcgcgaatccctgtacctggcggatgaagtgtttatgtccggtacggcggcagaaatcacgccagtgcgcagcgtagacggtattcaggttggcgaaggccgttgtggcccggttaccaaacgcattcagcaagccttcttcggcctcttcactggcgaaaccgaagataaatggggctggttagatcaagttaatcaataa

SEQ ID NO: 32 - DNA, 930 bp, Unknown
  ilvE
atgaccacgaagaaagctgattacatttggttcaatggggagatggttcgctgggaagacgcgaaggtgcatgtgatgtcgcacgcgctgcactatggcacttcggtttttgaaggcatccgttgctacgactcgcacaaaggaccggttgtattccgccatcgtgagcatatgcagcgtctgcatgactccgccaaaatctatcgcttcccggtttcgcagagcattgatgagctgatggaagcttgtcgtgacgtgatccgcaaaaacaatctcaccagcgcctatatcatcccgctgatcttcgtcggtgatgttggcatgggagtaaacccgccagcgggatactcaaccgacgtgattatcgctgctttcccgtggggagcgtatctgggcgcagaagcgctggagcaggggatcgatgcgatggtttcctcctggaaccgcgcagcaccaaacaccatcccgacggcggcaaaagccggtggtaactacctctcttccctgctggtgggtagcgaagcgcgccgccacggttatcaggaaggtatcgcgctggatgtgaacggttatatctctgaaggcgcaggcgaaaacctgtttgaagtgaaagatggtgtgctgttcaccccaccgttcacctcctccgcgctgccgggtattacccgtgatgccatcatcaaactggcgaaagagctgggaattgaagtacgtgagcaggtgctgtcgcgcgaatccctgtacctggcggatgaagtgtttatgtccggtacggcggcagaaatcacgccagtgcgcagcgtagacggtattcaggttggcgaaggccgttgtggcccggttaccaaacgcattcagcaagccttcttcggcctcttcactggcgaaaccgaagataaatggggctggttagatcaagttaatcaataa

SEQ ID NO: 33 - DNA, 930 bp, Unknown
  ilvE
atgaccacgaagaaagctgattacatttggttcaatggggagatggttcgctgggaagacgcgaaggtgcatgtgatgtcgcacgcgctgcactatggcacttcggtttttgaaggcatccgttgctacgactcgcacaaaggaccggttgtattccgccatcgtgagcatatgcagcgtctgcatgactccgccaaaatctatcgcttcccggtttcgcagagcattgatgagctgatggaagcttgtcgtgacgtgatccgcaaaaacaatctcaccagcgcctatatccgtccgctgatcttcgtcggtgatgttggcatgggagtaaacccgccagcgggatactcaaccgacgtgattatcgctgctttcccgtggggagcgtatctgggcgcagaagcgctggagcaggggatcgatgcgatggtttcctcctggaaccgcgcagcaccaaacaccatcccgacggcggcaaaagccggtggtaactacctctcttccctgctggtgggtagcgaagcgcgccgccacggttatcaggaaggtatcgcgctggatgtgaacggttatatctctgaaggcgcaggcgaaaacctgtttgaagtgaaagatggtgtgctgttcaccccaccgttcacctcctccgcgctgccgggtattacccgtgatgccatcatcaaactggcgaaagagctgggaattgaagtacgtgagcaggtgctgtcgcgcgaatccctgtacctggcggatgaagtgtttatggtgggtacggcggcagaaatcacgccagtgcgcagcgtagacggtattcaggttggcgaaggccgttgtggcccggttaccaaacgcattcagcaagccttcttcggcctcttcactggcgaaaccgaagataaatggggctggttagatcaagttaatcaataa

SEQ ID NO: 34 - DNA, 930 bp, Unknown
  ilvE
atgaccacgaagaaagctgattacatttggttcaatggggagatggttcgctgggaagacgcgaaggtgcatgtgatgtcgcacgcgctgctgtatggcacttcggtttttgaaggcatccgttgctacgactcgcacaaaggaccggttgtattccgccatcgtgagcatatgcagcgtctgcatgactccgccaaaatctatcgcttcccggtttcgcagagcattgatgagctgatggaagcttgtcgtgacgtgatccgcaaaaacaatctcaccagcgcctatatcatcccgctgatcttcgtcggtgatgttggcatgggagtaaacccgccagcgggatactcaaccgacgtgattatcgctgctttcccgtggggagcgtatctgggcgcagaagcgctggagcaggggatcgatgcgatggtttcctcctggaaccgcgcagcaccaaacaccatcccgacggcggcaaaagccggtggtaactacctctcttccctgctggtgggtagcgaagcgcgccgccacggttatcaggaaggtatcgcgctggatgtgaacggttatatctctgaaggcgcaggcgaaaacctgtttgaagtgaaagatggtgtgctgttcaccccaccgttcacctcctccgcgctgccgggtattacccgtgatgccatcatcaaactggcgaaagagctgggaattgaagtacgtgagcaggtgctgtcgcgcgaatccctgtacctggcggatgaagtgtttatgtccggtacggcggcagaaatcacgccagtgcgcagcgtagacggtattcaggttggcgaaggccgttgtggcccggttaccaaacgcattcagcaagccttcttcggcctcttcactggcgaaaccgaagataaatggggctggttagatcaagttaatcaataa

SEQ ID NO: 35 - DNA, 930 bp, Unknown
  ilvE
atgaccacgaagaaagctgattacatttggttcaatggggagatggttcgctgggaagacgcgaaggtgcatgtgatgtcgcacgcgctgctgtatggcacttcggtttttgaaggcatccgttgctacgactcgcacaaaggaccggttgtattccgccatcgtgagcatatgcagcgtctgcatgactccgccaaaatctatcgcttcccggtttcgcagagcattgatgagctgatggaagcttgtcgtgacgtgatccgcaaaaacaatctcaccagcgcctatatccgtccgctgatcttcgtcggtgatgttggcatgggagtaaacccgccagcgggatactcaaccgacgtgattatcgctgctttcccgtggggagcgtatctgggcgcagaagcgctggagcaggggatcgatgcgatggtttcctcctggaaccgcgcagcaccaaacaccatcccgacggcggcaaaagccggtggtaactacctctcttccctgctggtgggtagcgaagcgcgccgccacggttatcaggaaggtatcgcgctggatgtgaacggttatatctctgaaggcgcaggcgaaaacctgtttgaagtgaaagatggtgtgctgttcaccccaccgttcacctcctccgcgctgccgggtattacccgtgatgccatcatcaaactggcgaaagagctgggaattgaagtacgtgagcaggtgctgtcgcgcgaatccctgtacctggcggatgaagtgtttatggtgggtacggcggcagaaatcacgccagtgcgcagcgtagacggtattcaggttggcgaaggccgttgtggcccggttaccaaacgcattcagcaagccttcttcggcctcttcactggcgaaaccgaagataaatggggctggttagatcaagttaatcaataa

SEQ ID NO: 36 - DNA, 930 bp, Unknown
  ilvE
atgaccacgaagaaagctgattacatttggttcaatggggagatggttcgctgggaagacgcgaaggtgcatgtgatgtcgcacgcgctgcactatggcacttcggtttttgaaggcatccgttgctacgactcgcacaaaggaccggttgtattccgccatcgtgagcatatgcagcgtctgcatgactccgccaaaatctatcgcttcccggtttcgcagagcattgatgagctgatggaagcttgtcgtgacgtgatccgcaaaaacaatctcaccagcgcctatatcatcccgctgatcttcgtcggtgatgttggcatgggagtaaacccgccagcgggatactcaaccgacgtgattatcgctgctttcccgtggggagcgtatctgggcgcagaagcgctggagcaggggatcgatgcgatggtttcctcctggaaccgcgcagcaccaaacaccatcccgacggcggcaaaagccggtggtaactacctctcttccctgctggtgggtagcgaagcgcgccgccacggttatcaggaaggtatcgcgctggatgtgaacggttatatctctgaaggcgcaggcgaaaacctgtttgaagtgaaagatggtgtgctgttcaccccaccgttcacctcctccgcgctgccgggtattacccgtgatgccatcatcaaactggcgaaagagctgggaattgaagtacgtgagcaggtgctgtcgcgcgaatccctgtacctggcggatgaagtgtttatggtgggtacggcggcagaaatcacgccagtgcgcagcgtagacggtattcaggttggcgaaggccgttgtggcccggttaccaaacgcattcagcaagccttcttcggcctcttcactggcgaaaccgaagataaatggggctggttagatcaagttaatcaataa

SEQ ID NO: 37 - protein, 436 aa, Unknown
  ilvA
MSETYVSEKSPGVMASGAELIRAADIQTAQARISSVIAPTPLQYCPRLSEETGAEIYLKREDLQDVRSYKIRGALNSGAQLTQEQRDAGIVAASAGNHAQGVAYVCKSLGVQGRIYVPVQTPKQKRDRIMVHGGEFVSLVVTGNNFDEASAAAHEDAERTGATLIEPFDARNTVIGQGTVAAEILSQLTSMGKSADHVMVPVGGGGLLAGVVSYMADMAPRTAIVGIEPAGAASMQAALHNGGPITLETVDPFVDGAAVKRVGDLNYTIVEKNQGRVHMMSATEGAVCTEMLDLYQNEGIIAEPAGALSIAGLKEMSFAPGSVVVCIISGGNNDVLRYAEIAERSLVHRGLKHYFLVNFPQKPGQLRHFLEDILGPDDDITLFEYLKRNNRETGTALVGIHLSEASGLDSLLERMEESAIDSRRLEPGTPEYEYLT